European Patent Specification EP 3 797 787 B9, published October 4, 2023. Title: Zyklische, Amyloid-Beta-bindende Peptide und deren Verwendung. Applicant: Forschungszentrum Juelich GmbH. The sequence listing filed with the application follows.

SEQUENCE LISTING (11 sequences)

SEQ ID NO: 1 - protein, 24 aa, Artificial Sequence
  D-Peptid, cRD2D3
PTLHTHNRRRRRRPRTRLHTHRNR

SEQ ID NO: 2 - protein, 24 aa, Artificial Sequence
  D-Peptide, cD3D3
RPRTRLHTHRNRRPRTRLHTHRNR

SEQ ID NO: 3 - protein, 12 aa, Artificial Sequence
  D-Peptide, cRD2
PTLHTHNRRRRR

SEQ ID NO: 4 - protein, 24 aa, Artificial Sequence
  D-Peptide, cRD2RD2
PTLHTHNRRRRRPTLHTHNRRRRR

SEQ ID NO: 5 - protein, 13 aa, Artificial Sequence
  D-Peptide, cD3r
RPRTRLHTHRNRR

SEQ ID NO: 6 - protein, 13 aa, Artificial Sequence
  D-Peptide, cD3p
RPRTRLHTHRNRP

SEQ ID NO: 7 - protein, 13 aa, Artificial Sequence
  D-Peptide, cD3a
RPRTRLHTHRNRA

SEQ ID NO: 8 - protein, 12 aa, Artificial Sequence
  D-Peptide, cD3
RPRTRLHTHRNR

SEQ ID NO: 9 - protein, 12 aa, Artificial Sequence
  D-Peptide, cDB3
RPITRLRTHQNR

SEQ ID NO: 10 - protein, 24 aa, Artificial Sequence
  D-Peptide, cDB3DB3
RPITRLRTHQNRRPITRLRTHQNR

SEQ ID NO: 11 - protein, 12 aa, Artificial Sequence
  D-Peptide, cD3(p2k)
RKRTRLHTHRNR